European Patent Specification EP 3 699 181 B1, published March 1, 2023. Title: CRYSTALLINE FORM OF (S)-N-(5-((R)-2-(2,5-DIFLUOROPHENYL)-PYRROLIDIN-1-YL)-PYRAZOLO[l,5-A]PYRIMIDIN-3-YL)-3-HYDROXYPYRROLIDINE-1-CARBOXAMIDE HYDROGEN SULFATE. Applicant: Array Biopharma, Inc. The sequence listing filed with the application follows.

SEQUENCE LISTING (4 sequences)

SEQ ID NO: 1 - DNA, 18 bp, Artificial Sequence
  synthetic oligonucleotide
gagggcgagctgcatgat

SEQ ID NO: 2 - DNA, 20 bp, Artificial Sequence
  synthetic oligonucleotide
cggcgcttgatgtggtgaac

SEQ ID NO: 3 - protein, 9 aa, Artificial Sequence
  LMNA (exon 2)
HDLRGQVAK

SEQ ID NO: 4 - protein, 9 aa, Artificial Sequence
  NTRK1 (exon 11)
VSVAVGLAV